European Patent Specification EP 3 310 381 B1, published June 7, 2023. Title: IMMUNOGENIC COMPOSITIONS. Applicant: GlaxoSmithKline Biologicals S.A. The sequence listing filed with the application follows.

SEQUENCE LISTING (67 sequences)

SEQ ID NO: 1 - DNA, 36 bp, Artificial
  Shigella sonnei
actcgagctctgtagttgatttgacagttgacatcc

SEQ ID NO: 2 - DNA, 41 bp, Artificial
  Shigella sonnei
ctaacccgggcactatattatcagtaagtggttgataaacc

SEQ ID NO: 3 - DNA, 26 bp, Artificial
  Shigella sonnei
ctaacccgggcgtgttgatgtcctgc

SEQ ID NO: 4 - DNA, 31 bp, Artificial
  Shigella sonnei
acgcgtcgacagttcagttcaggctgtacgc

SEQ ID NO: 5 - DNA, 34 bp, Artificial
  Shigella sonnei
ctaacccgggcaagcaactctatgtcggtggaat

SEQ ID NO: 6 - DNA, 29 bp, Artificial
  Shigella sonnei
tatcaagcttggcaaggccaatacacagc

SEQ ID NO: 7 - DNA, 35 bp, Artificial
  Shigella sonnei
tatcaagcttagggttagagtgtctcgtttttgta

SEQ ID NO: 8 - DNA, 28 bp, Artificial
  Shigella sonnei
ctaacccgggccagaccagaactattcc

SEQ ID NO: 9 - DNA, 36 bp, Artificial
  Shigella flexneri
ctagtctagaaacccgggcaattgtatgtattgtcg

SEQ ID NO: 10 - DNA, 27 bp, Artificial
  Shigella flexneri
actcgagctcccgtcatcatccaacgc

SEQ ID NO: 11 - DNA, 29 bp, Artificial
  Shigella flexneri
actcgagctcatccgatatacgttcgccc

SEQ ID NO: 12 - DNA, 31 bp, Artificial
  Shigella flexneri
acgcgtcgacctcagtaatcagggttctttg

SEQ ID NO: 13 - DNA, 30 bp, Artificial
  Shigella flexneri
ctaacccgggtaaatctcccctgccggatg

SEQ ID NO: 14 - DNA, 31 bp, Artificial
  Shigella flexneri
acgcgtcgaccctgtaatctcaggtcaaatg

SEQ ID NO: 15 - DNA, 30 bp, Artificial
  Shigella flexneri
ctaacccgggtaaatctcccatgccggatg

SEQ ID NO: 16 - DNA, 36 bp, Artificial
  Shigella flexneri
ctagtctagaaacccgggtgatagtgtagcggcaca

SEQ ID NO: 17 - DNA, 27 bp, Artificial
  Shigella flexneri
actcgagctcgtgagcaaagccagctg

SEQ ID NO: 18 - DNA, 27 bp, Artificial
  Shigella flexneri
acgcgtcgacctcggtgtggaaattgg

SEQ ID NO: 19 - DNA, 29 bp, Artificial
  Shigella flexneri
ctaacccgggcaacgtacttactctaccg

SEQ ID NO: 20 - DNA, 31 bp, Artificial
  Shigella flexneri
accggaattcgtgtaacactggcatggtgta

SEQ ID NO: 21 - DNA, 31 bp, Artificial
  Shigella flexneri
catgccattgtagcaatccgctgttggtgcg

SEQ ID NO: 22 - DNA, 35 bp, Artificial
  Shigella flexneri
agcttgatatcagagtgtgttgatagtgcagtatc

SEQ ID NO: 23 - DNA, 34 bp, Artificial
  Shigella flexneri
agcttgatatcacctctttagcttcttggaagct

SEQ ID NO: 24 - DNA, 31 bp, Artificial
  Shigella flexneri
agcttgatatctgtgacggaagatcacttcg

SEQ ID NO: 25 - DNA, 31 bp, Artificial
  Shigella flexneri
agcttgatatcgggcaccaataactgcctta

SEQ ID NO: 26 - DNA, 24 bp, Artificial
  Shigella flexneri
cggcatcagaataatacaagcagc

SEQ ID NO: 27 - DNA, 19 bp, Artificial
  Shigella flexneri
aggtgtaccgtgctctggg

SEQ ID NO: 28 - DNA, 24 bp, Artificial
  Shigella flexneri
gtcacaggtaacatgactctggag

SEQ ID NO: 29 - DNA, 25 bp, Artificial
  Shigella flexneri
ccatgtgtgaatactaccttcaccc

SEQ ID NO: 30 - DNA, 25 bp, Artificial
  Shigella flexneri
gttttgcctcattcaagatatcacc

SEQ ID NO: 31 - DNA, 23 bp, Artificial
  Shigella flexneri
tgacgatggtttgtcaggattgc

SEQ ID NO: 32 - DNA, 23 bp, Artificial
  Shigella flexneri
cgccaaagttccgtgatcccatt

SEQ ID NO: 33 - DNA, 23 bp, Artificial
  Shigella flexneri
ctcttcgatgatctccagccctt

SEQ ID NO: 34 - DNA, 23 bp, Artificial
  Shigella flexneri
cacgtcttgagcgattgtgtagg

SEQ ID NO: 35 - DNA, 23 bp, Artificial
  Shigella flexneri
gacatgggaattagccatggtcc

SEQ ID NO: 36 - DNA, 19 bp, Artificial
  Shigella flexneri
caattggtctgttcgccgc

SEQ ID NO: 37 - DNA, 21 bp, Artificial
  Shigella flexneri
ctaccgcacctgaatcaacca

SEQ ID NO: 38 - DNA, 70 bp, Artificial
  Shigella flexneri
accgccaggcgtttaccgttagcgagagcaacaaggggtaagccatggccgtgtaggctggagctgcttc

SEQ ID NO: 39 - DNA, 70 bp, Artificial
  Shigella flexneri
acccgctctctttcaagcaagggaaacgcagatgtttagataggctgcgtcatatgaatatcctccttag

SEQ ID NO: 40 - DNA, 70 bp, Artificial
  Shigella flexneri
acaatacatacaattgcccgtataggttgaaaaacaggattgatatgacggtgtaggctggagctgcttc

SEQ ID NO: 41 - DNA, 70 bp, Artificial
  Shigella flexneri
atgccggatgccattctgaagcatccggcatgggagatttaatagcgtgacatatgaatatcctccttag

SEQ ID NO: 42 - DNA, 70 bp, Artificial
  Shigella flexneri
actatcaccagattgatttttgccttatccgaaactggaaaagcatggaagtgtaggctggagctgcttc

SEQ ID NO: 43 - DNA, 70 bp, Artificial
  Shigella flexneri
ttttatttgatgggataaagatctttgcgcttatacggctggatttcgcccatatgaatatcctccttag

SEQ ID NO: 44 - DNA, 21 bp, Artificial
  Shigella flexneri
cgatagggatgttgccaggtt

SEQ ID NO: 45 - DNA, 22 bp, Artificial
  Shigella flexneri
ctatcggcacgcacctcattta

SEQ ID NO: 46 - DNA, 24 bp, Artificial
  Shigella flexneri
ctttcccctgtttactggtttaca

SEQ ID NO: 47 - DNA, 17 bp, Artificial
  Shigella flexneri
tgtccgcgctggcaatg

SEQ ID NO: 48 - DNA, 20 bp, Artificial
  Shigella flexneri
aacccgcgtcgaactaatcc

SEQ ID NO: 49 - DNA, 45 bp, Artificial
  Shigella flexneri
cctacacaatcgctcaagacgtgcgtttccatgcttttccagttt

SEQ ID NO: 50 - DNA, 47 bp, Artificial
  Shigella flexneri
ggaccatggctaattcccatgtccccatcaaataaaaaagcctctcg

SEQ ID NO: 51 - DNA, 20 bp, Artificial
  Shigella flexneri
atcccgagcatcaacgtttc

SEQ ID NO: 52 - DNA, 19 bp, Artificial
  Shigella flexneri
gcgcagtacccagaaggat

SEQ ID NO: 53 - DNA, 46 bp, Artificial
  Shigella flexneri
cctacacaatcgctcaagacgtgggtggagaacttgggtagattcg

SEQ ID NO: 54 - DNA, 46 bp, Artificial
  Shigella flexneri
ggaccatggctaattcccatgtcccttcacgctattaaatctccca

SEQ ID NO: 55 - DNA, 22 bp, Artificial
  Shigella flexneri
tgactacatctacaccagccct

SEQ ID NO: 56 - DNA, 20 bp, Artificial
  Shigella flexneri
gcgtactttggttggtcgtg

SEQ ID NO: 57 - DNA, 18 bp, Artificial
  Shigella flexneri
aacgaagggcaccagaca

SEQ ID NO: 58 - DNA, 22 bp, Artificial
  Shigella flexneri
ggttatgatggctacggtggta

SEQ ID NO: 59 - DNA, 22 bp, Artificial
  Shigella flexneri
gtttatagtccttctgcgccca

SEQ ID NO: 60 - DNA, 20 bp, Artificial
  Shigella flexneri
aacccgcgtcgaactaatcc

SEQ ID NO: 61 - DNA, 45 bp, Artificial; identical to SEQ ID NO: 49
  Shigella flexneri

SEQ ID NO: 62 - DNA, 47 bp, Artificial; identical to SEQ ID NO: 50
  Shigella flexneri

SEQ ID NO: 63 - DNA, 20 bp, Artificial
  Shigella flexneri
atcccgagcatcaacgtttc

SEQ ID NO: 64 - DNA, 19 bp, Artificial
  Shigella flexneri
gcgcagtacccagaaggat

SEQ ID NO: 65 - DNA, 46 bp, Artificial; identical to SEQ ID NO: 53
  Shigella flexneri

SEQ ID NO: 66 - DNA, 46 bp, Artificial; identical to SEQ ID NO: 54
  Shigella flexneri

SEQ ID NO: 67 - DNA, 22 bp, Artificial
  Shigella flexneri
tgactacatctacaccagccct